European Patent Application EP 4 752 223 A2, published June 3, 2026. Title: CANCER-TARGETED, VIRUS-ENCODED, REGULATABLE T (CATVERT) OR NK CELL (CATVERN) LINKERS. Applicant: RESEARCH INSTITUTE AT NATIONWIDE CHILDREN'S HOSPITAL. Application IP OFFICE CODE APPLICATION NUMBER. The sequence listing filed with the application follows.

SEQUENCE LISTING (71 sequences)

SEQ ID NO: 1 - DNA, 24 bp, synthetic construct
  misc_feature 1..24: note = Description of Artificial Sequence: Synthetic oligonucleotide
  misc_difference 4: note = a, c, t, g, unknown or other
  misc_difference 8: note = a, c, t, g, unknown or other
  misc_difference 12: note = a, c, t, g, unknown or other
  misc_difference 16: note = a, c, t, g, unknown or other
  misc_difference 20: note = a, c, t, g, unknown or other
  misc_difference 24: note = a, c, t, g, unknown or other
  source 1..24: mol_type = other DNA
taantagntgantagntaantgan

SEQ ID NO: 2 - DNA, 24 bp, synthetic construct
  misc_feature 1..24: note = Description of Artificial Sequence: Synthetic oligonucleotide
  source 1..24: mol_type = other DNA
taattagttgattagttaattgat

SEQ ID NO: 3 - protein, 162 aa, unidentified
  REGION 1..162: note = Description of Unknown: IL-21 sequence
MRSSPGNMERIVICLMVIFLGTLVHKSSSQGQDRHMIRMRQLIDIVDQLKNYVNDLVPEFLPAPEDVETNCEWSAFSCFQKAQLKSANTGNNERIINVSIKKLKRKPPSTNAGRRQKHRLTCPSCDSYEKKPPKEFLERFKSLLQKMIHQHLSSRTHGSEDS

SEQ ID NO: 4 - DNA, 486 bp, unidentified
  misc_feature 1..486: note = Description of Unknown: IL-21 sequence
  source 1..486: mol_type = unassigned DNA
atgagaagcagccccggcaacatggagagaatcgtgatctgcctgatggtgatcttcctgggcaccctggtgcacaagagcagcagccagggccaggacagacacatgatcagaatgagacagctgatcgacatcgtggaccagctgaagaactacgtgaacgacctggtgcccgagttcctgcccgcccccgaggacgtggagaccaactgcgagtggagcgccttcagctgcttccagaaggcccagctgaagagcgccaacaccggcaacaacgagagaatcatcaacgtgagcatcaagaagctgaagagaaagccccccagcaccaacgccggcagaagacagaagcacagactgacctgccccagctgcgacagctacgagaagaagccccccaaggagttcctggagagattcaagagcctgctgcagaagatgatccaccagcacctgagcagcagaacccacggcagcgaggacagc

SEQ ID NO: 5 - protein, 274 aa, unidentified
  REGION 1..274: note = Description of Unknown: MICA sequence
EPHSLRYNLTVLSWDGSVQSGFLAEVHLDGQPFLRYDRQKCRAKPQGQWAEDVLGNKTWDRETRDLTGNGKDLRMTLAHIKDQKEGLHSLQEIRVCEIHEDNSTRSSQHFYYDGELFLSQNLETEEWTVPQSSRAQTLAMNVRNFLKEDAMKTKTHYHAMHADCLQELRRYLESSVVLRRTVPPMVNVTRSEASEGNITVTCRASSFYPRNIILTWRQDGVSLSHDTQQWGDVLPDGNGTYQTWVATRICRGEEQRFTCYMEHSGNHSTHPVPS

SEQ ID NO: 6 - DNA, 822 bp, unidentified
  misc_feature 1..822: note = Description of Unknown: MICA sequence
  source 1..822: mol_type = unassigned DNA
gagccccacagtcttcgttataacctcacggtgctgtcctgggatggatctgtgcagtcagggtttcttgctgaggtacatctggatggtcagcccttcctgcgctatgacaggcagaaatgcagggcaaagccccagggacagtgggcagaagatgtcctgggaaataagacatgggacagagagaccagggacttgacagggaacggaaaggacctcaggatgaccctggctcatatcaaggaccagaaagaaggcttgcattccctccaggagattagggtctgtgagatccatgaagacaacagcaccaggagctcccagcatttctactacgatggggagctcttcctctcccaaaacctggagactgaggaatggacagtgccccagtcctccagagctcagaccttggccatgaacgtcaggaatttcttgaaggaagatgccatgaagaccaagacacactatcacgctatgcatgcagactgcctgcaggaactacggcgatatctagaatccagcgtagtcctgaggagaacagtgccccccatggtgaatgtcacccgcagcgaggcctcagagggcaacatcaccgtgacatgcagggcttccagcttctatccccggaatatcatactgacctggcgtcaggatggggtatctttgagccacgacacccagcagtggggggatgtcctgcctgatgggaatggaacctaccagacctgggtggccaccaggatttgccgaggagaggagcagaggttcacctgctacatggaacacagcgggaatcacagcactcaccctgtgccctct

SEQ ID NO: 7 - protein, 274 aa, synthetic construct
  REGION 1..274: note = Description of Artificial Sequence: Synthetic polypeptide
EPHSLRYNLTVLSWDGSVQSGFLAEVHLDGQPFLRCDRQKCRAKPQGQWAEDVLGNKTWDRETRDLTGNGKDLRMTLAHIKDQKEGLHSLQEIRVCEIHEDNSTRSSQHFYYDGELFLSQNLETEEWTMPQSSRAQTLAMNIRNFLKEDAMKTKTHYHAMHADCLQELRRYLKSGVVLRRTVPPMVNVTRSEASEGNITVTCRASGFYPWNITLSWRQDGVSLSHDTQQWGDVLPDGNGTYQTWVATRICQGEEQRFTCYMEHSGNHSTHPVPS

SEQ ID NO: 8 - DNA, 822 bp, synthetic construct
  misc_feature 1..822: note = Description of Artificial Sequence: Synthetic polynucleotide
  source 1..822: mol_type = other DNA
gagccccacagtcttcgttataacctcacggtgctgtcctgggatggatctgtgcagtcagggtttctcgctgaggtacatctggatggtcagcccttcctgcgctgtgacaggcagaaatgcagggcaaagccccagggacagtgggcagaagatgtcctgggaaataagacatgggacagagagaccagggacttgacagggaacggaaaggacctcaggatgaccctggctcatatcaaggaccagaaagaaggcttgcattccctccaggagattagggtctgtgagatccatgaagacaacagcaccaggagctcccagcatttctactacgatggggagctcttcctctcccaaaacctggagactgaggaatggacaatgccccagtcctccagagctcagaccttggccatgaacatcaggaatttcttgaaggaagatgccatgaagaccaagacacactatcacgctatgcatgcagactgcctgcaggaactacggcgatatctaaaatccggcgtagtcctgaggagaacagtgccccccatggtgaatgtcacccgcagcgaggcctcagagggcaacattaccgtgacatgcagggcttctggcttctatccctggaatatcacactgagctggcgtcaggatggggtatctttgagccacgacacccagcagtggggggatgtcctgcctgatgggaatggaacctaccagacctgggtggccaccaggatttgccaaggagaggagcagaggttcacctgctacatggaacacagcgggaatcacagcactcaccctgtgccctct

SEQ ID NO: 9 - protein, 15 aa, synthetic construct
  REGION 1..15: note = Description of Artificial Sequence: Synthetic peptide
GGGGSGGGGSGGGGS

SEQ ID NO: 10 - DNA, 45 bp, synthetic construct
  misc_feature 1..45: note = Description of Artificial Sequence: Synthetic oligonucleotide
  source 1..45: mol_type = other DNA
ggcggcggcggcagcggcggcggcggcagcggcggcggcggcagc

SEQ ID NO: 11 - protein, 732 aa, synthetic construct
  REGION 1..732: note = Description of Artificial Sequence: Synthetic polypeptide
MWWRLWWLLLLLLLLWPMVWAARSSPGNMERIVICLMVIFLGTLVHKSSSQGQDRHMIRMRQLIDIVDQLKNYVNDLVPEFLPAPEDVETNCEWSAFSCFQKAQLKSANTGNNERIINVSIKKLKRKPPSTNAGRRQKHRLTCPSCDSYEKKPPKEFLERFKSLLQKMIHQHLSSRTHGSEDSGGGGSGGGGSGGGGSEPHSLRYNLTVLSWDGSVQSGFLAEVHLDGQPFLRCDRQKCRAKPQGQWAEDVLGNKTWDRETRDLTGNGKDLRMTLAHIKDQKEGLHSLQEIRVCEIHEDNSTRSSQHFYYDGELFLSQNLETEEWTMPQSSRAQTLAMNIRNFLKEDAMKTKTHYHAMHADCLQELRRYLKSGVVLRRTVPPMVNVTRSEASEGNITVTCRASGFYPWNITLSWRQDGVSLSHDTQQWGDVLPDGNGTYQTWVATRICQGEEQRFTCYMEHSGNHSTHPVPSGGGGSGGGGSGGGGSQVQLQQSGPELVKPGASVKISCKTSGYKFTEYTMHWVKQSHGKCLEWIGGINPNNGGTNYNQKFKGKATLTVDKSSSTAYMELRSLTSEDSAVYYCARDTTVPYAYWGQGTTVTVSSGGGGSGGGGSGGGGSDIELTQSPAIMSASPGEKVTMTCSASSSISYMHWYQQKPGTSPKRWIYDTSKLASSVPARFSGSGSGTSYSLTISSMEAEDAATYYCHQRSSYPLTFGCGTKLEIKRASTKGP

SEQ ID NO: 12 - DNA, 2199 bp, synthetic construct
  misc_feature 1..2199: note = Description of Artificial Sequence: Synthetic polynucleotide
  source 1..2199: mol_type = other DNA
atgtggtggagactgtggtggctgctgctgctgctgctgctgctgtggcccatggtgtgggccgccagaagcagccccggcaacatggagagaatcgtgatctgcctgatggtgatcttcctgggcaccctggtgcacaagagcagcagccagggccaggacagacacatgatcagaatgagacagctgatcgacatcgtggaccagctgaagaactacgtgaacgacctggtgcccgagttcctgcccgcccccgaggacgtggagaccaactgcgagtggagcgccttcagctgcttccagaaggcccagctgaagagcgccaacaccggcaacaacgagagaatcatcaacgtgagcatcaagaagctgaagagaaagccccccagcaccaacgccggcagaagacagaagcacagactgacctgccccagctgcgacagctacgagaagaagccccccaaggagttcctggagagattcaagagcctgctgcagaagatgatccaccagcacctgagcagcagaacccacggcagcgaggacagcggcggcggcggcagcggcggcggcggcagcggcggcggcggcagcgagccccacagtcttcgttataacctcacggtgctgtcctgggatggatctgtgcagtcagggtttctcgctgaggtacatctggatggtcagcccttcctgcgctgtgacaggcagaaatgcagggcaaagccccagggacagtgggcagaagatgtcctgggaaataagacatgggacagagagaccagggacttgacagggaacggaaaggacctcaggatgaccctggctcatatcaaggaccagaaagaaggcttgcattccctccaggagattagggtctgtgagatccatgaagacaacagcaccaggagctcccagcatttctactacgatggggagctcttcctctcccaaaacctggagactgaggaatggacaatgccccagtcctccagagctcagaccttggccatgaacatcaggaatttcttgaaggaagatgccatgaagaccaagacacactatcacgctatgcatgcagactgcctgcaggaactacggcgatatctaaaatccggcgtagtcctgaggagaacagtgccccccatggtgaatgtcacccgcagcgaggcctcagagggcaacattaccgtgacatgcagggcttctggcttctatccctggaatatcacactgagctggcgtcaggatggggtatctttgagccacgacacccagcagtggggggatgtcctgcctgatgggaatggaacctaccagacctgggtggccaccaggatttgccaaggagaggagcagaggttcacctgctacatggaacacagcgggaatcacagcactcaccctgtgccctctggcggcggcggcagcggcggcggcggcagcggcggcggcggcagccaggtgcagctgcagcagagcggccccgagctggtgaagcccggcgccagcgtgaagatcagctgcaagaccagcggctacaagttcaccgagtacaccatgcactgggtgaagcagagccacggcaagtgcctggagtggatcggcggcatcaaccccaacaacggcggcaccaactacaaccagaagttcaagggcaaggccaccctgaccgtggacaagagcagcagcaccgcctacatggagctgagaagcctgaccagcgaggacagcgccgtgtactactgcgccagagacaccaccgtgccctacgcctactggggccagggcaccaccgtgaccgtgagcagcggcggcggcggcagcggcggcggcggcagcggcggcggcggcagcgacatcgagctgacccagagccccgccatcatgagcgccagccccggcgagaaggtgaccatgacctgcagcgccagcagcagcatcagctacatgcactggtaccagcagaagcccggcaccagccccaagagatggatctacgacaccagcaagctggccagcagcgtgcccgccagattcagcggcagcggcagcggcaccagctacagcctgaccatcagcagcatggaggccgaggacgccgccacctactactgccaccagagaagcagctaccccctgaccttcggctgcggcaccaagctggagatcaagagagccagcaccaagggcccctag

SEQ ID NO: 13 - protein, 572 aa, synthetic construct
  REGION 1..572: note = Description of Artificial Sequence: Synthetic polypeptide
MWWRLWWLLLLLLLLWPMVWAAQVQLQQSGPELVKPGASVKISCKTSGYKFTEYTMHWVKQSHGKCLEWIGGINPNNGGTNYNQKFKGKATLTVDKSSSTAYMELRSLTSEDSAVYYCARDTTVPYAYWGQGTTVTVSSGGGGSGGGGSGGGGSDIELTQSPAIMSASPGEKVTMTCSASSSISYMHWYQQKPGTSPKRWIYDTSKLASSVPARFSGSGSGTSYSLTISSMEAEDAATYYCHQRSSYPLTFGCGTKLEIKRASTKGPGGGGSGGGGSGGGGSQVQLVQSGGGVVQPGRSLRLSCKASGYTFTRYTMHWVRQAPGKGLEWIGYINPSRGYTNYNQKFKDRFTISRDNSKNTAFLQMDSLRPEDTGVYFCARYYDDHYCLDYWGQGTPVTVSSGGGGSGGGGSGGGGSDIQMTQSPSSLSASVGDRVTITCSASSSVSYMNWYQQTPGKAPKRWIYDTSKLASGVPSRFSGSGSGTDYTFTISSLQPEDIATYYCQQWSSNPFTFGQGTKLQITRTPLGDTTHTSGMVSKLSQLQTELLAALLESGLSKEALIQALGEGSGGAP

SEQ ID NO: 14 - DNA, 1719 bp, synthetic construct
  misc_feature 1..1719: note = Description of Artificial Sequence: Synthetic polynucleotide
  source 1..1719: mol_type = other DNA
atgtggtggagactgtggtggctgctgctgctgctgctgctgctgtggcccatggtgtgggccgcccaggtgcagctgcagcagagcggccccgagctggtgaagcccggcgccagcgtgaagatcagctgcaagaccagcggctacaagttcaccgagtacaccatgcactgggtgaagcagagccacggcaagtgcctggagtggatcggcggcatcaaccccaacaacggcggcaccaactacaaccagaagttcaagggcaaggccaccctgaccgtggacaagagcagcagcaccgcctacatggagctgagaagcctgaccagcgaggacagcgccgtgtactactgcgccagagacaccaccgtgccctacgcctactggggccagggcaccaccgtgaccgtgagcagcggcggcggcggcagcggcggcggcggcagcggcggcggcggcagcgacatcgagctgacccagagccccgccatcatgagcgccagccccggcgagaaggtgaccatgacctgcagcgccagcagcagcatcagctacatgcactggtaccagcagaagcccggcaccagccccaagagatggatctacgacaccagcaagctggccagcagcgtgcccgccagattcagcggcagcggcagcggcaccagctacagcctgaccatcagcagcatggaggccgaggacgccgccacctactactgccaccagagaagcagctaccccctgaccttcggctgcggcaccaagctggagatcaagagagccagcaccaagggccccggcggcggcggcagcggcggcggcggcagcggcggcggcggcagccaggtgcagctggtgcagagcggcggcggcgtggtgcagcccggcagaagcctgagactgagctgcaaggccagcggctacaccttcaccagatacaccatgcactgggtgagacaggcccccggcaagggcctggagtggatcggctacatcaaccccagcagaggctacaccaactacaaccagaagttcaaggacagattcaccatcagcagagacaacagcaagaacaccgccttcctgcagatggacagcctgagacccgaggacaccggcgtgtacttctgcgccagatactacgacgaccactactgcctggactactggggccagggcacccccgtgaccgtgagcagcggcggcggcggcagcggcggcggcggcagcggcggcggcggcagcgacatccagatgacccagagccccagcagcctgagcgccagcgtgggcgacagagtgaccatcacctgcagcgccagcagcagcgtgagctacatgaactggtaccagcagacccccggcaaggcccccaagagatggatctacgacaccagcaagctggccagcggcgtgcccagcagattcagcggcagcggcagcggcaccgactacaccttcaccatcagcagcctgcagcccgaggacatcgccacctactactgccagcagtggagcagcaaccccttcaccttcggccagggcaccaagctgcagatcaccagaacccccctgggcgacaccacccacaccagcggcatggtgagcaagctgagccagctgcagaccgagctgctggccgccctgctggagagcggcctgagcaaggaggccctgatccaggccctgggcgagggcagcggcggcgccccctag

SEQ ID NO: 15 - protein, 575 aa, synthetic construct
  REGION 1..575: note = Description of Artificial Sequence: Synthetic polypeptide
MWWRLWWLLLLLLLLWPMVWAADIQLTQSPASLAVSLGQRATISCKASQSVDYDGDSYLNWYQQIPGQPPKLLIYDASNLVSGIPPRFSGSGSGTDFTLNIHPVEKVDAATYHCQQSTEDPWTFGGGTKLEIKGGGGSGGGGSGGGGSQVQLQQSGAELVRPGSSVKISCKASGYAFSSYWMNWVKQRPGQGLEWIGQIWPGDGDTNYNGKFKGKATLTADESSSTAYMQLSSLASEDSAVYFCARRETTTVGRYYYAMDYWGQGTTVTVSSGGGGSDIKLQQSGAELARPGASVKMSCKTSGYTFTRYTMHWVKQRPGQGLEWIGYINPSRGYTNYNQKFKDKATLTTDKSSSTAYMQLSSLTSEDSAVYYCARYYDDHYCLDYWGQGTTLTVSSVEGGSGGSGGSGGSGGVDDIQLTQSPAIMSASPGEKVTMTCRASSSVSYMNWYQQKSGTSPKRWIYDTSKVASGVPYRFSGSGSGTSYSLTISSMEAEDAATYYCQQWSSNPLTFGAGTKLELKHHHHHHTPLGDTTHTSGMVSKLSQLQTELLAALLESGLSKEALIQALGEGSGGAP

SEQ ID NO: 16 - DNA, 1727 bp, synthetic construct
  misc_feature 1..1727: note = Description of Artificial Sequence: Synthetic polynucleotide
  source 1..1727: mol_type = other DNA
atgtggtggagactgtggtggctgctgctgctgctgctgctgctgtggcccatggtgtgggccgccgacatccagctgacccagagccccgccagcctggccgtgagcctgggccagagagccaccatcagctgcaaggccagccagagcgtggactacgacggcgacagctacctgaactggtaccagcagatccccggccagccccccaagctgctgatctacgacgccagcaacctggtgagcggcatcccccccagattcagcggcagcggcagcggcaccgacttcaccctgaacatccaccccgtggagaaggtggacgccgccacctaccactgccagcagagcaccgaggacccctggaccttcggcggcggcaccaagctggagatcaagggcggcggcggcagcggcggcggcggcagcggcggcggcggcagccaggtgcagctgcagcagagcggcgccgagctggtgagacccggcagcagcgtgaagatcagctgcaaggccagcggctacgccttcagcagctactggatgaactgggtgaagcagagacccggccagggcctggagtggatcggccagatctggcccggcgacggcgacaccaactacaacggcaagttcaagggcaaggccaccctgaccgccgacgagagcagcagcaccgcctacatgcagctgagcagcctggccagcgaggacagcgccgtgtacttctgcgccagaagagagaccaccaccgtgggcagatactactacgccatggactactggggccagggcaccaccgtgaccgtgagcagcggcggcggcggcagcgacatcaagctgcagcagagcggcgccgagctggccagacccggcgccagcgtgaagatgagctgcaagaccagcggctacaccttcaccagatacaccatgcactgggtgaagcagagacccggccagggcctggagtggatcggctacatcaaccccagcagaggctacaccaactacaaccagaagttcaaggacaaggccaccctgaccaccgacaagagcagcagcaccgcctacatgcagctgagcagcctgaccagcgaggacagcgccgtgtactactgcgccagatactacgacgaccactactgcctggactactggggccagggcaccaccctgaccgtgagcagcgtggagggcggcagcggcggcagcggcggcagcggcggcagcggcggcgtggacgacatccagctgacccagagccccgccatcatgagcgccagccccggcgagaaggtgaccatgacctgcagagccagcagcagcgtgagctacatgaactggtaccagcagaagagcggcaccagccccaagagatggatctacgacaccagcaaggtggccagcggcgtgccctacagattcagcggcagcggcagcggcaccagctacagcctgaccatcagcagcatggaggccgaggacgccgccacctactactgccagcagtggagcagcaaccccctgaccttcggcgccggcaccaagctggagctgaagcaccaccaccaccaccacacccccctgggcgacaccacccacaccagcggcatggtgagcaagctgagccagctgcagaccgagctgctggccgccctgctggagagcggcctgagcaaggaggccctgatccaggccctgggcgagggcagcggcggcgcccccta

SEQ ID NO: 17 - DNA, 122 bp, synthetic construct
  misc_feature 1..122: note = Description of Artificial Sequence: Synthetic polynucleotide
  source 1..122: mol_type = other DNA
gcctgctgaaaatgactgaatataaacttgtggtagttggagctggtggcgtaggcaagagtgccttgacgatacagctaattcagaatcattttgtggacgaatatgatccaacaatagag

SEQ ID NO: 18 - DNA, 122 bp, synthetic construct
  misc_feature 1..122: note = Description of Artificial Sequence: Synthetic polynucleotide
  source 1..122: mol_type = other DNA
gcctgctgaaataattagctgagtagataagtgatgttggagctggtggcgtaggcaagagtgccttgacgatacagctaattcagaatcattttgtggacgaatatgatccaacaatagag

SEQ ID NO: 19 - DNA, 150 bp, synthetic construct
  misc_feature 1..150: note = Description of Artificial Sequence: Synthetic polynucleotide
  source 1..150: mol_type = other DNA
gtacggagcggaccacccctcctgggcccctgcccgggtcccgaccctctttgccggcgccgggcggggccggcggagtatttgatagtgtattaaccttatgtgtgacatgttctaatatagtcacattttcattatttttattataag

SEQ ID NO: 20 - DNA, 150 bp, synthetic construct
  misc_feature 1..150: note = Description of Artificial Sequence: Synthetic polynucleotide
  source 1..150: mol_type = other DNA
gtaaatcttgttttaatatgcatattactggtgcaggaccattctttgatacagataaaggtttctctgaccattttgagttgtatataacaccttttttgaagtaaaaggtgcactgtaataatccagactgtgtttctcccttctcag

SEQ ID NO: 21 - DNA, 422 bp, synthetic construct
  misc_feature 1..422: note = Description of Artificial Sequence: Synthetic polynucleotide
  source 1..422: mol_type = other DNA
gtacggagcggaccacccctcctgggcccctgcccgggtcccgaccctctttgccggcgccgggcggggccggcggagtatttgatagtgtattaaccttatgtgtgacatgttctaatatagtcacattttcattatttttattataaggcctgctgaaataattagctgagtagataagtgatgttggagctggtggcgtaggcaagagtgccttgacgatacagctaattcagaatcattttgtggacgaatatgatccaacaatagaggtaaatcttgttttaatatgcatattactggtgcaggaccattctttgatacagataaaggtttctctgaccattttgagttgtatataacaccttttttgaagtaaaaggtgcactgtaataatccagactgtgtttctcccttctcag

SEQ ID NO: 22 - DNA, 1722 bp, synthetic construct
  misc_feature 1..1722: note = Description of Artificial Sequence: Synthetic polynucleotide
  source 1..1722: mol_type = other DNA
atgtggtggagactgtggtggctgctgctgctgctgctgctgctgtggcccatggtgtgggccgccgcccaggtgcagctgcagcagagcggccccgagctggtgaagcccggcgccagcgtgaagatcagctgcaagaccagcggctacaagttcaccgagtacaccatgcactgggtgaagcagagccacggcaagtgcctggagtggatcggcggcatcaaccccaacaacggcggcaccaactacaaccagaagttcaagggcaaggccaccctgaccgtggacaagagcagcagcaccgcctacatggagctgagaagcctgaccagcgaggacagcgccgtgtactactgcgccagagacaccaccgtgccctacgcctactggggccagggcaccaccgtgaccgtgagcagcggcggcggcggcagcggcggcggcggcagcggcggcggcggcagcgacatcgagctgacccagagccccgccatcatgagcgccagccccggcgagaaggtgaccatgacctgcagcgccagcagcagcatcagctacatgcactggtaccagcagaagcccggcaccagccccaagagatggatctacgacaccagcaagctggccagcagcgtgcccgccagattcagcggcagcggcagcggcaccagctacagcctgaccatcagcagcatggaggccgaggacgccgccacctactactgccaccagagaagcagctaccccctgaccttcggctgcggcaccaagctggagatcaagagagccagcaccaagggccccggcggcggcggcagcggcggcggcggcagcggcggcggcggcagccaggtgcagctggtgcagagcggcggcggcgtggtgcagcccggcagaagcctgagactgagctgcaaggccagcggctacaccttcaccagatacaccatgcactgggtgagacaggcccccggcaagggcctggagtggatcggctacatcaaccccagcagaggctacaccaactacaaccagaagttcaaggacagattcaccatcagcagagacaacagcaagaacaccgccttcctgcagatggacagcctgagacccgaggacaccggcgtgtacttctgcgccagatactacgacgaccactactgcctggactactggggccagggcacccccgtgaccgtgagcagcggcggcggcggcagcggcggcggcggcagcggcggcggcggcagcgacatccagatgacccagagccccagcagcctgagcgccagcgtgggcgacagagtgaccatcacctgcagcgccagcagcagcgtgagctacatgaactggtaccagcagacccccggcaaggcccccaagagatggatctacgacaccagcaagctggccagcggcgtgcccagcagattcagcggcagcggcagcggcaccgactacaccttcaccatcagcagcctgcagcccgaggacatcgccacctactactgccagcagtggagcagcaaccccttcaccttcggccagggcaccaagctgcagatcaccagaacccccctgggcgacaccacccacaccagcggcatggtgagcaagctgagccagctgcagaccgagctgctggccgccctgctggagagcggcctgagcaaggaggccctgatccaggccctgggcgagggcagcggcggcgccccctag

SEQ ID NO: 23 - DNA, 2144 bp, synthetic construct
  misc_feature 1..2144: note = Description of Artificial Sequence: Synthetic polynucleotide
  source 1..2144: mol_type = other DNA
atgtggtggagactgtggtggctgctgctgctgctgctgctgctgtggcccatggtgtgggccgccgcccaggtgcagctgcagcagagcggccccgagctggtgaagcccggcgccagcgtgaagatcagctgcaagaccagcggctacaagttcaccgagtacaccatgcactgggtgaagcagagccacggcaagtgcctggagtggatcggcggcatcaaccccaacaacggcggcaccaactacaaccagaagttcaaggtacggagcggaccacccctcctgggcccctgcccgggtcccgaccctctttgccggcgccgggcggggccggcggagtatttgatagtgtattaaccttatgtgtgacatgttctaatatagtcacattttcattatttttattataaggcctgctgaaataattagctgagtagataagtgatgttggagctggtggcgtaggcaagagtgccttgacgatacagctaattcagaatcattttgtggacgaatatgatccaacaatagaggtaaatcttgttttaatatgcatattactggtgcaggaccattctttgatacagataaaggtttctctgaccattttgagttgtatataacaccttttttgaagtaaaaggtgcactgtaataatccagactgtgtttctcccttctcagggcaaggccaccctgaccgtggacaagagcagcagcaccgcctacatggagctgagaagcctgaccagcgaggacagcgccgtgtactactgcgccagagacaccaccgtgccctacgcctactggggccagggcaccaccgtgaccgtgagcagcggcggcggcggcagcggcggcggcggcagcggcggcggcggcagcgacatcgagctgacccagagccccgccatcatgagcgccagccccggcgagaaggtgaccatgacctgcagcgccagcagcagcatcagctacatgcactggtaccagcagaagcccggcaccagccccaagagatggatctacgacaccagcaagctggccagcagcgtgcccgccagattcagcggcagcggcagcggcaccagctacagcctgaccatcagcagcatggaggccgaggacgccgccacctactactgccaccagagaagcagctaccccctgaccttcggctgcggcaccaagctggagatcaagagagccagcaccaagggccccggcggcggcggcagcggcggcggcggcagcggcggcggcggcagccaggtgcagctggtgcagagcggcggcggcgtggtgcagcccggcagaagcctgagactgagctgcaaggccagcggctacaccttcaccagatacaccatgcactgggtgagacaggcccccggcaagggcctggagtggatcggctacatcaaccccagcagaggctacaccaactacaaccagaagttcaaggacagattcaccatcagcagagacaacagcaagaacaccgccttcctgcagatggacagcctgagacccgaggacaccggcgtgtacttctgcgccagatactacgacgaccactactgcctggactactggggccagggcacccccgtgaccgtgagcagcggcggcggcggcagcggcggcggcggcagcggcggcggcggcagcgacatccagatgacccagagccccagcagcctgagcgccagcgtgggcgacagagtgaccatcacctgcagcgccagcagcagcgtgagctacatgaactggtaccagcagacccccggcaaggcccccaagagatggatctacgacaccagcaagctggccagcggcgtgcccagcagattcagcggcagcggcagcggcaccgactacaccttcaccatcagcagcctgcagcccgaggacatcgccacctactactgccagcagtggagcagcaaccccttcaccttcggccagggcaccaagctgcagatcaccagaacccccctgggcgacaccacccacaccagcggcatggtgagcaagctgagccagctgcagaccgagctgctggccgccctgctggagagcggcctgagcaaggaggccctgatccaggccctgggcgagggcagcggcggcgccccctag

SEQ ID NO: 24 - DNA, 30 bp, synthetic construct
  misc_feature 1..30: note = Description of Artificial Sequence: Synthetic oligonucleotide
  source 1..30: mol_type = other DNA
aatatgatccaacaatagaggtaaatcttg

SEQ ID NO: 25 - DNA, 30 bp, synthetic construct
  misc_feature 1..30: note = Description of Artificial Sequence: Synthetic oligonucleotide
  source 1..30: mol_type = other DNA
gatccaacaatagaggtaaatcttgtttta

SEQ ID NO: 26 - DNA, 51 bp, synthetic construct
  misc_feature 1..51: note = Description of Artificial Sequence: Synthetic oligonucleotide
  source 1..51: mol_type = other DNA
aatatgatccaacaatagaggtaaatcttgttttaatatgcatattactgg

SEQ ID NO: 27 - DNA, 30 bp, synthetic construct
  misc_feature 1..30: note = Description of Artificial Sequence: Synthetic oligonucleotide
  source 1..30: mol_type = other DNA
caagatttacctctattgttggatcatatt

SEQ ID NO: 28 - DNA, 30 bp, synthetic construct
  misc_feature 1..30: note = Description of Artificial Sequence: Synthetic oligonucleotide
  source 1..30: mol_type = other DNA
taaaacaagatttacctctattgttggatc

SEQ ID NO: 29 - protein, 527 aa, synthetic construct
  REGION 1..527: note = Description of Artificial Sequence: Synthetic polypeptide
MWWRLWWLLLLLLLLWPMVWAAADIQLTQSPASLAVSLGQRATISCKASQSVDYDGDSYLNWYQQIPGQPPKLLIYDASNLVSGIPPRFSGSGSGTDFTLNIHPVEKVDAATYHCQQSTEDPWTFGGGTKLEIKGGGGSGGGGSGGGGSQVQLQQSGAELVRPGSSVKISCKASGYAFSSYWMNWVKQRPGQGLEWIGQIWPGDGDTNYNGKFKGKATLTADESSSTAYMQLSSLASEDSAVYFCARRETTTVGRYYYAMDYWGQGTTVTVSSGGGGSDIKLQQSGAELARPGASVKMSCKTSGYTFTRYTMHWVKQRPGQGLEWIGYINPSRGYTNYNQKFKDKATLTTDKSSSTAYMQLSSLTSEDSAVYYCARYYDDHYCLDYWGQGTTLTVSSVEGGSGGSGGSGGSGGVDDIQLTQSPAIMSASPGEKVTMTCRASSSVSYMNWYQQKSGTSPKRWIYDTSKVASGVPYRFSGSGSGTSYSLTISSMEAEDAATYYCQQWSSNPLTFGAGTKLELKHHHHHH

SEQ ID NO: 30 - DNA, 1584 bp, synthetic construct
  misc_feature 1..1584: note = Description of Artificial Sequence: Synthetic polynucleotide
  source 1..1584: mol_type = other DNA
atgtggtggagactgtggtggctgctgctgctgctgctgctgctgtggcccatggtgtgggccgccgccgacatccagctgacccagagccccgccagcctggccgtgagcctgggccagagagccaccatcagctgcaaggccagccagagcgtggactacgacggcgacagctacctgaactggtaccagcagatccccggccagccccccaagctgctgatctacgacgccagcaacctggtgagcggcatcccccccagattcagcggcagcggcagcggcaccgacttcaccctgaacatccaccccgtggagaaggtggacgccgccacctaccactgccagcagagcaccgaggacccctggaccttcggcggcggcaccaagctggagatcaagggcggcggcggcagcggcggcggcggcagcggcggcggcggcagccaggtgcagctgcagcagagcggcgccgagctggtgagacccggcagcagcgtgaagatcagctgcaaggccagcggctacgccttcagcagctactggatgaactgggtgaagcagagacccggccagggcctggagtggatcggccagatctggcccggcgacggcgacaccaactacaacggcaagttcaagggcaaggccaccctgaccgccgacgagagcagcagcaccgcctacatgcagctgagcagcctggccagcgaggacagcgccgtgtacttctgcgccagaagagagaccaccaccgtgggcagatactactacgccatggactactggggccagggcaccaccgtgaccgtgagcagcggcggcggcggcagcgacatcaagctgcagcagagcggcgccgagctggccagacccggcgccagcgtgaagatgagctgcaagaccagcggctacaccttcaccagatacaccatgcactgggtgaagcagagacccggccagggcctggagtggatcggctacatcaaccccagcagaggctacaccaactacaaccagaagttcaaggacaaggccaccctgaccaccgacaagagcagcagcaccgcctacatgcagctgagcagcctgaccagcgaggacagcgccgtgtactactgcgccagatactacgacgaccactactgcctggactactggggccagggcaccaccctgaccgtgagcagcgtggagggcggcagcggcggcagcggcggcagcggcggcagcggcggcgtggacgacatccagctgacccagagccccgccatcatgagcgccagccccggcgagaaggtgaccatgacctgcagagccagcagcagcgtgagctacatgaactggtaccagcagaagagcggcaccagccccaagagatggatctacgacaccagcaaggtggccagcggcgtgccctacagattcagcggcagcggcagcggcaccagctacagcctgaccatcagcagcatggaggccgaggacgccgccacctactactgccagcagtggagcagcaaccccctgaccttcggcgccggcaccaagctggagctgaagcaccaccaccaccaccactag

SEQ ID NO: 31 - DNA, 1581 bp, synthetic construct
  misc_feature 1..1581: note = Description of Artificial Sequence: Synthetic polynucleotide
  source 1..1581: mol_type = other DNA
atgtggtggagactgtggtggctgctgctgctgctgctgctgctgtggcccatggtgtgggccgccgacatccagctgacccagagccccgccagcctggccgtgagcctgggccagagagccaccatcagctgcaaggccagccagagcgtggactacgacggcgacagctacctgaactggtaccagcagatccccggccagccccccaagctgctgatctacgacgccagcaacctggtgagcggcatcccccccagattcagcggcagcggcagcggcaccgacttcaccctgaacatccaccccgtggagaaggtggacgccgccacctaccactgccagcagagcaccgaggacccctggaccttcggcggcggcaccaagctggagatcaagggcggcggcggcagcggcggcggcggcagcggcggcggcggcagccaggtgcagctgcagcagagcggcgccgagctggtgagacccggcagcagcgtgaagatcagctgcaaggccagcggctacgccttcagcagctactggatgaactgggtgaagcagagacccggccagggcctggagtggatcggccagatctggcccggcgacggcgacaccaactacaacggcaagttcaagggcaaggccaccctgaccgccgacgagagcagcagcaccgcctacatgcagctgagcagcctggccagcgaggacagcgccgtgtacttctgcgccagaagagagaccaccaccgtgggcagatactactacgccatggactactggggccagggcaccaccgtgaccgtgagcagcggcggcggcggcagcgacatcaagctgcagcagagcggcgccgagctggccagacccggcgccagcgtgaagatgagctgcaagaccagcggctacaccttcaccagatacaccatgcactgggtgaagcagagacccggccagggcctggagtggatcggctacatcaaccccagcagaggctacaccaactacaaccagaagttcaaggacaaggccaccctgaccaccgacaagagcagcagcaccgcctacatgcagctgagcagcctgaccagcgaggacagcgccgtgtactactgcgccagatactacgacgaccactactgcctggactactggggccagggcaccaccctgaccgtgagcagcgtggagggcggcagcggcggcagcggcggcagcggcggcagcggcggcgtggacgacatccagctgacccagagccccgccatcatgagcgccagccccggcgagaaggtgaccatgacctgcagagccagcagcagcgtgagctacatgaactggtaccagcagaagagcggcaccagccccaagagatggatctacgacaccagcaaggtggccagcggcgtgccctacagattcagcggcagcggcagcggcaccagctacagcctgaccatcagcagcatggaggccgaggacgccgccacctactactgccagcagtggagcagcaaccccctgaccttcggcgccggcaccaagctggagctgaagcaccaccaccaccaccactag

SEQ ID NO: 32 - DNA, 1578 bp, synthetic construct
  misc_feature 1..1578: note = Description of Artificial Sequence: Synthetic polynucleotide
  source 1..1578: mol_type = other DNA
atgtggtggagactgtggtggctgctgctgctgctgctgctgctgtggcccatggtgtgggccgacatccagctgacccagagccccgccagcctggccgtgagcctgggccagagagccaccatcagctgcaaggccagccagagcgtggactacgacggcgacagctacctgaactggtaccagcagatccccggccagccccccaagctgctgatctacgacgccagcaacctggtgagcggcatcccccccagattcagcggcagcggcagcggcaccgacttcaccctgaacatccaccccgtggagaaggtggacgccgccacctaccactgccagcagagcaccgaggacccctggaccttcggcggcggcaccaagctggagatcaagggcggcggcggcagcggcggcggcggcagcggcggcggcggcagccaggtgcagctgcagcagagcggcgccgagctggtgagacccggcagcagcgtgaagatcagctgcaaggccagcggctacgccttcagcagctactggatgaactgggtgaagcagagacccggccagggcctggagtggatcggccagatctggcccggcgacggcgacaccaactacaacggcaagttcaagggcaaggccaccctgaccgccgacgagagcagcagcaccgcctacatgcagctgagcagcctggccagcgaggacagcgccgtgtacttctgcgccagaagagagaccaccaccgtgggcagatactactacgccatggactactggggccagggcaccaccgtgaccgtgagcagcggcggcggcggcagcgacatcaagctgcagcagagcggcgccgagctggccagacccggcgccagcgtgaagatgagctgcaagaccagcggctacaccttcaccagatacaccatgcactgggtgaagcagagacccggccagggcctggagtggatcggctacatcaaccccagcagaggctacaccaactacaaccagaagttcaaggacaaggccaccctgaccaccgacaagagcagcagcaccgcctacatgcagctgagcagcctgaccagcgaggacagcgccgtgtactactgcgccagatactacgacgaccactactgcctggactactggggccagggcaccaccctgaccgtgagcagcgtggagggcggcagcggcggcagcggcggcagcggcggcagcggcggcgtggacgacatccagctgacccagagccccgccatcatgagcgccagccccggcgagaaggtgaccatgacctgcagagccagcagcagcgtgagctacatgaactggtaccagcagaagagcggcaccagccccaagagatggatctacgacaccagcaaggtggccagcggcgtgccctacagattcagcggcagcggcagcggcaccagctacagcctgaccatcagcagcatggaggccgaggacgccgccacctactactgccagcagtggagcagcaaccccctgaccttcggcgccggcaccaagctggagctgaagcaccaccaccaccaccactag

SEQ ID NO: 33 - DNA, 1518 bp, synthetic construct
  misc_feature 1..1518: note = Description of Artificial Sequence: Synthetic polynucleotide
  source 1..1518: mol_type = other DNA
atggacatccagctgacccagagccccgccagcctggccgtgagcctgggccagagagccaccatcagctgcaaggccagccagagcgtggactacgacggcgacagctacctgaactggtaccagcagatccccggccagccccccaagctgctgatctacgacgccagcaacctggtgagcggcatcccccccagattcagcggcagcggcagcggcaccgacttcaccctgaacatccaccccgtggagaaggtggacgccgccacctaccactgccagcagagcaccgaggacccctggaccttcggcggcggcaccaagctggagatcaagggcggcggcggcagcggcggcggcggcagcggcggcggcggcagccaggtgcagctgcagcagagcggcgccgagctggtgagacccggcagcagcgtgaagatcagctgcaaggccagcggctacgccttcagcagctactggatgaactgggtgaagcagagacccggccagggcctggagtggatcggccagatctggcccggcgacggcgacaccaactacaacggcaagttcaagggcaaggccaccctgaccgccgacgagagcagcagcaccgcctacatgcagctgagcagcctggccagcgaggacagcgccgtgtacttctgcgccagaagagagaccaccaccgtgggcagatactactacgccatggactactggggccagggcaccaccgtgaccgtgagcagcggcggcggcggcagcgacatcaagctgcagcagagcggcgccgagctggccagacccggcgccagcgtgaagatgagctgcaagaccagcggctacaccttcaccagatacaccatgcactgggtgaagcagagacccggccagggcctggagtggatcggctacatcaaccccagcagaggctacaccaactacaaccagaagttcaaggacaaggccaccctgaccaccgacaagagcagcagcaccgcctacatgcagctgagcagcctgaccagcgaggacagcgccgtgtactactgcgccagatactacgacgaccactactgcctggactactggggccagggcaccaccctgaccgtgagcagcgtggagggcggcagcggcggcagcggcggcagcggcggcagcggcggcgtggacgacatccagctgacccagagccccgccatcatgagcgccagccccggcgagaaggtgaccatgacctgcagagccagcagcagcgtgagctacatgaactggtaccagcagaagagcggcaccagccccaagagatggatctacgacaccagcaaggtggccagcggcgtgccctacagattcagcggcagcggcagcggcaccagctacagcctgaccatcagcagcatggaggccgaggacgccgccacctactactgccagcagtggagcagcaaccccctgaccttcggcgccggcaccaagctggagctgaagcaccaccaccaccaccactag

SEQ ID NO: 34-39 - skipped (6 entries)

SEQ ID NO: 40 - DNA, 2144 bp, synthetic construct
  misc_feature 1..2144: note = Description of Artificial Sequence: Synthetic polynucleotide
  source 1..2144: mol_type = other DNA
atgtggtggagactgtggtggctgctgctgctgctgctgctgctgtggcccatggtgtgggccgccgcccaggtgcagctgcagcagagcggccccgagctggtgaagcccggcgccagcgtgaagatcagctgcaagaccagcggctacaagttcaccgagtacaccatgcactgggtgaagcagagccacggcaagtgcctggagtggatcggcggcatcaaccccaacaacggcggcaccaactacaaccagaagttcaaggtacggagcggaccacccctcctgggcccctgcccgggtcccgaccctctttgccggcgccgggcggggccggcggagtatttgatagtgtattaaccttatgtgtgacatgttctaatatagtcacattttccttcttttttttttcaggcctgctgaaataattagctgagtagataagtgatgttggagctggtggcgtaggcaagagtgccttgacgatacagctaattcagaatcattttgtggacgaatatgatccaacaatagaggtaaatcttgttttaatatgcatattactggtgcaggaccattctttgatacagataaaggtttctctgaccattttgagttgtatataacaccttttttgaagtaaaaggtgcactgtaataatccagactgtgtttctcccttctcagggcaaggccaccctgaccgtggacaagagcagcagcaccgcctacatggagctgagaagcctgaccagcgaggacagcgccgtgtactactgcgccagagacaccaccgtgccctacgcctactggggccagggcaccaccgtgaccgtgagcagcggcggcggcggcagcggcggcggcggcagcggcggcggcggcagcgacatcgagctgacccagagccccgccatcatgagcgccagccccggcgagaaggtgaccatgacctgcagcgccagcagcagcatcagctacatgcactggtaccagcagaagcccggcaccagccccaagagatggatctacgacaccagcaagctggccagcagcgtgcccgccagattcagcggcagcggcagcggcaccagctacagcctgaccatcagcagcatggaggccgaggacgccgccacctactactgccaccagagaagcagctaccccctgaccttcggctgcggcaccaagctggagatcaagagagccagcaccaagggccccggcggcggcggcagcggcggcggcggcagcggcggcggcggcagccaggtgcagctggtgcagagcggcggcggcgtggtgcagcccggcagaagcctgagactgagctgcaaggccagcggctacaccttcaccagatacaccatgcactgggtgagacaggcccccggcaagggcctggagtggatcggctacatcaaccccagcagaggctacaccaactacaaccagaagttcaaggacagattcaccatcagcagagacaacagcaagaacaccgccttcctgcagatggacagcctgagacccgaggacaccggcgtgtacttctgcgccagatactacgacgaccactactgcctggactactggggccagggcacccccgtgaccgtgagcagcggcggcggcggcagcggcggcggcggcagcggcggcggcggcagcgacatccagatgacccagagccccagcagcctgagcgccagcgtgggcgacagagtgaccatcacctgcagcgccagcagcagcgtgagctacatgaactggtaccagcagacccccggcaaggcccccaagagatggatctacgacaccagcaagctggccagcggcgtgcccagcagattcagcggcagcggcagcggcaccgactacaccttcaccatcagcagcctgcagcccgaggacatcgccacctactactgccagcagtggagcagcaaccccttcaccttcggccagggcaccaagctgcagatcaccagaacccccctgggcgacaccacccacaccagcggcatggtgagcaagctgagccagctgcagaccgagctgctggccgccctgctggagagcggcctgagcaaggaggccctgatccaggccctgggcgagggcagcggcggcgccccctag

SEQ ID NO: 41 - DNA, 2144 bp, synthetic construct
  misc_feature 1..2144: note = Description of Artificial Sequence: Synthetic polynucleotide
  source 1..2144: mol_type = other DNA
atgtggtggagactgtggtggctgctgctgctgctgctgctgctgtggcccatggtgtgggccgccgcccaggtgcagctgcagcagagcggccccgagctggtgaagcccggcgccagcgtgaagatcagctgcaagaccagcggctacaagttcaccgagtacaccatgcactgggtgaagcagagccacggcaagtgcctggagtggatcggcggcatcaaccccaacaacggcggcaccaactacaaccagaagttcaaggtacggagcggaccacccctcctgggcccctgcccgggtcccgaccctctttgccggcgccgggcggggccggcggagtatttgatagtgtattaaccttatgtgtgacatgttctaatatagtcacattttccttcttttttttttaaggcctgctgaaataattagctgagtagataagtgatgttggagctggtggcgtaggcaagagtgccttgacgatacagctaattcagaatcattttgtggacgaatatgatccaacaatagaggtaaatcttgttttaatatgcatattactggtgcaggaccattctttgatacagataaaggtttctctgaccattttgagttgtatataacaccttttttgaagtaaaaggtgcactgtaataatccagactgtgtttctcccttctcagggcaaggccaccctgaccgtggacaagagcagcagcaccgcctacatggagctgagaagcctgaccagcgaggacagcgccgtgtactactgcgccagagacaccaccgtgccctacgcctactggggccagggcaccaccgtgaccgtgagcagcggcggcggcggcagcggcggcggcggcagcggcggcggcggcagcgacatcgagctgacccagagccccgccatcatgagcgccagccccggcgagaaggtgaccatgacctgcagcgccagcagcagcatcagctacatgcactggtaccagcagaagcccggcaccagccccaagagatggatctacgacaccagcaagctggccagcagcgtgcccgccagattcagcggcagcggcagcggcaccagctacagcctgaccatcagcagcatggaggccgaggacgccgccacctactactgccaccagagaagcagctaccccctgaccttcggctgcggcaccaagctggagatcaagagagccagcaccaagggccccggcggcggcggcagcggcggcggcggcagcggcggcggcggcagccaggtgcagctggtgcagagcggcggcggcgtggtgcagcccggcagaagcctgagactgagctgcaaggccagcggctacaccttcaccagatacaccatgcactgggtgagacaggcccccggcaagggcctggagtggatcggctacatcaaccccagcagaggctacaccaactacaaccagaagttcaaggacagattcaccatcagcagagacaacagcaagaacaccgccttcctgcagatggacagcctgagacccgaggacaccggcgtgtacttctgcgccagatactacgacgaccactactgcctggactactggggccagggcacccccgtgaccgtgagcagcggcggcggcggcagcggcggcggcggcagcggcggcggcggcagcgacatccagatgacccagagccccagcagcctgagcgccagcgtgggcgacagagtgaccatcacctgcagcgccagcagcagcgtgagctacatgaactggtaccagcagacccccggcaaggcccccaagagatggatctacgacaccagcaagctggccagcggcgtgcccagcagattcagcggcagcggcagcggcaccgactacaccttcaccatcagcagcctgcagcccgaggacatcgccacctactactgccagcagtggagcagcaaccccttcaccttcggccagggcaccaagctgcagatcaccagaacccccctgggcgacaccacccacaccagcggcatggtgagcaagctgagccagctgcagaccgagctgctggccgccctgctggagagcggcctgagcaaggaggccctgatccaggccctgggcgagggcagcggcggcgccccctag

SEQ ID NO: 42 - DNA, 2143 bp, synthetic construct
  misc_feature 1..2143: note = Description of Artificial Sequence: Synthetic polynucleotide
  source 1..2143: mol_type = other DNA
atgtggtggagactgtggtggctgctgctgctgctgctgctgctgtggcccatggtgtgggccgccgcccaggtgcagctgcagcagagcggccccgagctggtgaagcccggcgccagcgtgaagatcagctgcaagaccagcggctacaagttcaccgagtacaccatgcactgggtgaagcagagccacggcaagtgcctggagtggatcggcggcatcaaccccaacaacggcggcaccaactacaaccagaagttcaaggtacggagcggaccacccctcctgggcccctgcccgggtcccgaccctctttgccggcgccgggcggggccggcggagtatttgatagtgtattaaccttatgtgtgacatgttctaatatagtcacattttccttctttttattataagcctgctgaaataattagctgagtagataagtgatgttggagctggtggcgtaggcaagagtgccttgacgatacagctaattcagaatcattttgtggacgaatatgatccaacaatagaggtaaatcttgttttaatatgcatattactggtgcaggaccattctttgatacagataaaggtttctctgaccattttgagttgtatataacaccttttttgaagtaaaaggtgcactgtaataatccagactgtgtttctcccttctcagggcaaggccaccctgaccgtggacaagagcagcagcaccgcctacatggagctgagaagcctgaccagcgaggacagcgccgtgtactactgcgccagagacaccaccgtgccctacgcctactggggccagggcaccaccgtgaccgtgagcagcggcggcggcggcagcggcggcggcggcagcggcggcggcggcagcgacatcgagctgacccagagccccgccatcatgagcgccagccccggcgagaaggtgaccatgacctgcagcgccagcagcagcatcagctacatgcactggtaccagcagaagcccggcaccagccccaagagatggatctacgacaccagcaagctggccagcagcgtgcccgccagattcagcggcagcggcagcggcaccagctacagcctgaccatcagcagcatggaggccgaggacgccgccacctactactgccaccagagaagcagctaccccctgaccttcggctgcggcaccaagctggagatcaagagagccagcaccaagggccccggcggcggcggcagcggcggcggcggcagcggcggcggcggcagccaggtgcagctggtgcagagcggcggcggcgtggtgcagcccggcagaagcctgagactgagctgcaaggccagcggctacaccttcaccagatacaccatgcactgggtgagacaggcccccggcaagggcctggagtggatcggctacatcaaccccagcagaggctacaccaactacaaccagaagttcaaggacagattcaccatcagcagagacaacagcaagaacaccgccttcctgcagatggacagcctgagacccgaggacaccggcgtgtacttctgcgccagatactacgacgaccactactgcctggactactggggccagggcacccccgtgaccgtgagcagcggcggcggcggcagcggcggcggcggcagcggcggcggcggcagcgacatccagatgacccagagccccagcagcctgagcgccagcgtgggcgacagagtgaccatcacctgcagcgccagcagcagcgtgagctacatgaactggtaccagcagacccccggcaaggcccccaagagatggatctacgacaccagcaagctggccagcggcgtgcccagcagattcagcggcagcggcagcggcaccgactacaccttcaccatcagcagcctgcagcccgaggacatcgccacctactactgccagcagtggagcagcaaccccttcaccttcggccagggcaccaagctgcagatcaccagaacccccctgggcgacaccacccacaccagcggcatggtgagcaagctgagccagctgcagaccgagctgctggccgccctgctggagagcggcctgagcaaggaggccctgatccaggccctgggcgagggcagcggcggcgccccctag

SEQ ID NO: 43 - DNA, 2144 bp, synthetic construct
  misc_feature 1..2144: note = Description of Artificial Sequence: Synthetic polynucleotide
  source 1..2144: mol_type = other DNA
atgtggtggagactgtggtggctgctgctgctgctgctgctgctgtggcccatggtgtgggccgccgcccaggtgcagctgcagcagagcggccccgagctggtgaagcccggcgccagcgtgaagatcagctgcaagaccagcggctacaagttcaccgagtacaccatgcactgggtgaagcagagccacggcaagtgcctggagtggatcggcggcatcaaccccaacaacggcggcaccaactacaaccagaagttcaaggtacggagcggaccacccctcctgggcccctgcccgggtcccgaccctctttgccggcgccgggcggggccggcggagtatttgatagtgtattaaccttatgtgtgacatgttctaatatagtcacattttcattattttttttttcaggcctgctgaaataattagctgagtagataagtgatgttggagctggtggcgtaggcaagagtgccttgacgatacagctaattcagaatcattttgtggacgaatatgatccaacaatagaggtaaatcttgttttaatatgcatattactggtgcaggaccattctttgatacagataaaggtttctctgaccattttgagttgtatataacaccttttttgaagtaaaaggtgcactgtaataatccagactgtgtttctcccttctcagggcaaggccaccctgaccgtggacaagagcagcagcaccgcctacatggagctgagaagcctgaccagcgaggacagcgccgtgtactactgcgccagagacaccaccgtgccctacgcctactggggccagggcaccaccgtgaccgtgagcagcggcggcggcggcagcggcggcggcggcagcggcggcggcggcagcgacatcgagctgacccagagccccgccatcatgagcgccagccccggcgagaaggtgaccatgacctgcagcgccagcagcagcatcagctacatgcactggtaccagcagaagcccggcaccagccccaagagatggatctacgacaccagcaagctggccagcagcgtgcccgccagattcagcggcagcggcagcggcaccagctacagcctgaccatcagcagcatggaggccgaggacgccgccacctactactgccaccagagaagcagctaccccctgaccttcggctgcggcaccaagctggagatcaagagagccagcaccaagggccccggcggcggcggcagcggcggcggcggcagcggcggcggcggcagccaggtgcagctggtgcagagcggcggcggcgtggtgcagcccggcagaagcctgagactgagctgcaaggccagcggctacaccttcaccagatacaccatgcactgggtgagacaggcccccggcaagggcctggagtggatcggctacatcaaccccagcagaggctacaccaactacaaccagaagttcaaggacagattcaccatcagcagagacaacagcaagaacaccgccttcctgcagatggacagcctgagacccgaggacaccggcgtgtacttctgcgccagatactacgacgaccactactgcctggactactggggccagggcacccccgtgaccgtgagcagcggcggcggcggcagcggcggcggcggcagcggcggcggcggcagcgacatccagatgacccagagccccagcagcctgagcgccagcgtgggcgacagagtgaccatcacctgcagcgccagcagcagcgtgagctacatgaactggtaccagcagacccccggcaaggcccccaagagatggatctacgacaccagcaagctggccagcggcgtgcccagcagattcagcggcagcggcagcggcaccgactacaccttcaccatcagcagcctgcagcccgaggacatcgccacctactactgccagcagtggagcagcaaccccttcaccttcggccagggcaccaagctgcagatcaccagaacccccctgggcgacaccacccacaccagcggcatggtgagcaagctgagccagctgcagaccgagctgctggccgccctgctggagagcggcctgagcaaggaggccctgatccaggccctgggcgagggcagcggcggcgccccctag

SEQ ID NO: 44 - DNA, 1581 bp, synthetic construct; identical to SEQ ID NO: 31
  misc_feature 1..1581: note = Description of Artificial Sequence: Synthetic polynucleotide
  source 1..1581: mol_type = other DNA

SEQ ID NO: 45 - DNA, 2003 bp, synthetic construct
  misc_feature 1..2003: note = Description of Artificial Sequence: Synthetic polynucleotide
  source 1..2003: mol_type = other DNA
atgtggtggagactgtggtggctgctgctgctgctgctgctgctgtggcccatggtgtgggccgccgacatccagctgacccagagccccgccagcctggccgtgagcctgggccagagagccaccatcagctgcaaggccagccagagcgtggactacgacggcgacagctacctgaactggtaccagcagatccccggccagccccccaagctgctgatctacgacgccagcaacctggtgagcggcatcccccccagattcagcggcagcggcagcggcaccgacttcaccctgaacatccaccccgtggagaaggtacggagcggaccacccctcctgggcccctgcccgggtcccgaccctctttgccggcgccgggcggggccggcggagtatttgatagtgtattaaccttatgtgtgacatgttctaatatagtcacattttcattatttttattataaggcctgctgaaataattagctgagtagataagtgatgttggagctggtggcgtaggcaagagtgccttgacgatacagctaattcagaatcattttgtggacgaatatgatccaacaatagaggtaaatcttgttttaatatgcatattactggtgcaggaccattctttgatacagataaaggtttctctgaccattttgagttgtatataacaccttttttgaagtaaaaggtgcactgtaataatccagactgtgtttctcccttctcaggtggacgccgccacctaccactgccagcagagcaccgaggacccctggaccttcggcggcggcaccaagctggagatcaagggcggcggcggcagcggcggcggcggcagcggcggcggcggcagccaggtgcagctgcagcagagcggcgccgagctggtgagacccggcagcagcgtgaagatcagctgcaaggccagcggctacgccttcagcagctactggatgaactgggtgaagcagagacccggccagggcctggagtggatcggccagatctggcccggcgacggcgacaccaactacaacggcaagttcaagggcaaggccaccctgaccgccgacgagagcagcagcaccgcctacatgcagctgagcagcctggccagcgaggacagcgccgtgtacttctgcgccagaagagagaccaccaccgtgggcagatactactacgccatggactactggggccagggcaccaccgtgaccgtgagcagcggcggcggcggcagcgacatcaagctgcagcagagcggcgccgagctggccagacccggcgccagcgtgaagatgagctgcaagaccagcggctacaccttcaccagatacaccatgcactgggtgaagcagagacccggccagggcctggagtggatcggctacatcaaccccagcagaggctacaccaactacaaccagaagttcaaggacaaggccaccctgaccaccgacaagagcagcagcaccgcctacatgcagctgagcagcctgaccagcgaggacagcgccgtgtactactgcgccagatactacgacgaccactactgcctggactactggggccagggcaccaccctgaccgtgagcagcgtggagggcggcagcggcggcagcggcggcagcggcggcagcggcggcgtggacgacatccagctgacccagagccccgccatcatgagcgccagccccggcgagaaggtgaccatgacctgcagagccagcagcagcgtgagctacatgaactggtaccagcagaagagcggcaccagccccaagagatggatctacgacaccagcaaggtggccagcggcgtgccctacagattcagcggcagcggcagcggcaccagctacagcctgaccatcagcagcatggaggccgaggacgccgccacctactactgccagcagtggagcagcaaccccctgaccttcggcgccggcaccaagctggagctgaagcaccaccaccaccaccactag

SEQ ID NO: 46 - DNA, 2003 bp, synthetic construct
  misc_feature 1..2003: note = Description of Artificial Sequence: Synthetic polynucleotide
  source 1..2003: mol_type = other DNA
atgtggtggagactgtggtggctgctgctgctgctgctgctgctgtggcccatggtgtgggccgccgacatccagctgacccagagccccgccagcctggccgtgagcctgggccagagagccaccatcagctgcaaggccagccagagcgtggactacgacggcgacagctacctgaactggtaccagcagatccccggccagccccccaagctgctgatctacgacgccagcaacctggtgagcggcatcccccccagattcagcggcagcggcagcggcaccgacttcaccctgaacatccaccccgtggagaaggtacggagcggaccacccctcctgggcccctgcccgggtcccgaccctctttgccggcgccgggcggggccggcggagtatttgatagtgtattaaccttatgtgtgacatgttctaatatagtcacattttccttcttttttttttaaggcctgctgaaataattagctgagtagataagtgatgttggagctggtggcgtaggcaagagtgccttgacgatacagctaattcagaatcattttgtggacgaatatgatccaacaatagaggtaaatcttgttttaatatgcatattactggtgcaggaccattctttgatacagataaaggtttctctgaccattttgagttgtatataacaccttttttgaagtaaaaggtgcactgtaataatccagactgtgtttctcccttctcaggtggacgccgccacctaccactgccagcagagcaccgaggacccctggaccttcggcggcggcaccaagctggagatcaagggcggcggcggcagcggcggcggcggcagcggcggcggcggcagccaggtgcagctgcagcagagcggcgccgagctggtgagacccggcagcagcgtgaagatcagctgcaaggccagcggctacgccttcagcagctactggatgaactgggtgaagcagagacccggccagggcctggagtggatcggccagatctggcccggcgacggcgacaccaactacaacggcaagttcaagggcaaggccaccctgaccgccgacgagagcagcagcaccgcctacatgcagctgagcagcctggccagcgaggacagcgccgtgtacttctgcgccagaagagagaccaccaccgtgggcagatactactacgccatggactactggggccagggcaccaccgtgaccgtgagcagcggcggcggcggcagcgacatcaagctgcagcagagcggcgccgagctggccagacccggcgccagcgtgaagatgagctgcaagaccagcggctacaccttcaccagatacaccatgcactgggtgaagcagagacccggccagggcctggagtggatcggctacatcaaccccagcagaggctacaccaactacaaccagaagttcaaggacaaggccaccctgaccaccgacaagagcagcagcaccgcctacatgcagctgagcagcctgaccagcgaggacagcgccgtgtactactgcgccagatactacgacgaccactactgcctggactactggggccagggcaccaccctgaccgtgagcagcgtggagggcggcagcggcggcagcggcggcagcggcggcagcggcggcgtggacgacatccagctgacccagagccccgccatcatgagcgccagccccggcgagaaggtgaccatgacctgcagagccagcagcagcgtgagctacatgaactggtaccagcagaagagcggcaccagccccaagagatggatctacgacaccagcaaggtggccagcggcgtgccctacagattcagcggcagcggcagcggcaccagctacagcctgaccatcagcagcatggaggccgaggacgccgccacctactactgccagcagtggagcagcaaccccctgaccttcggcgccggcaccaagctggagctgaagcaccaccaccaccaccactag

SEQ ID NO: 47 - protein, 32 aa, Homo sapiens
MVSKLSQLQTELLAALLESGLSKEALIQALGE

SEQ ID NO: 48 - DNA, 96 bp, Homo sapiens
  source 1..96: mol_type = unassigned DNA
atggtgagcaagctgagccagctgcagaccgagctgctggccgccctgctggagagcggcctgagcaaggaggccctgatccaggccctgggcgag

SEQ ID NO: 49 - DNA, 313 bp, unidentified
  misc_feature 1..313: note = Description of Unknown: EFS promoter sequence
  source 1..313: mol_type = unassigned DNA
gtccgttatcaacttgaaaaagtggcaccgagtcggtgcttttttgaattcgctagctaggtcttgaaaggagtgggaattggctccggtgcccgtcagtgggcagagcgcacatcgcccacagtccccgagaagttggggggaggggtcggcaattgatccggtgcctagagaaggtggcgcggggtaaactgggaaagtgatgtcgtgtactggctccgcctttttcccgagggtgggggagaaccgtatataagtgcagtagtcgccgtgaacgttctttttcgcaacgggtttgccgccagaacacagg

SEQ ID NO: 50 - DNA, 597 bp, unidentified
  misc_feature 1..597: note = Description of Unknown: WPRE sequence
  source 1..597: mol_type = unassigned DNA
tcgacaatcaacctctggattacaaaatttgtgaaagattgactggtattcttaactatgttgctccttttacgctatgtggatacgctgctttaatgcctttgtatcatgctattgcttcccgtatggctttcattttctcctccttgtataaatcctggttgctgtctctttatgaggagttgtggcccgttgtcaggcaacgtggcgtggtgtgcactgtgtttgctgacgcaacccccactggttggggcattgccaccacctgtcagctcctttccgggactttcgctttccccctccctattgccacggcggaactcatcgccgcctgccttgcccgctgctggacaggggctcggctgttgggcactgacaattccgtggtgttgtcggggaagctgacgtcctttccatggctgctcgcctgtgttgccacctggattctgcgcgggacgtccttctgctacgtcccttcggccctcaatccagcggaccttccttcccgcggcctgctgccggctctgcggcctcttccgcgtcttcgccttcgccctcagacgagtcggatctccctttgggccgcctccccgcctg

SEQ ID NO: 51 - protein, 21 aa, synthetic construct
  REGION 1..21: note = Description of Artificial Sequence: Synthetic peptide
MWWRLWWLLLLLLLLWPMVWA

SEQ ID NO: 52 - DNA, 63 bp, synthetic construct
  misc_feature 1..63: note = Description of Artificial Sequence: Synthetic oligonucleotide
  source 1..63: mol_type = other DNA
atgtggtggagactgtggtggctgctgctgctgctgctgctgctgtggcccatggtgtgggcc

SEQ ID NO: 53 - protein, 22 aa, synthetic construct
  REGION 1..22: note = Description of Artificial Sequence: Synthetic peptide
MWWRLWWLLLLLLLLWPMVWAA

SEQ ID NO: 54 - DNA, 66 bp, synthetic construct
  misc_feature 1..66: note = Description of Artificial Sequence: Synthetic oligonucleotide
  source 1..66: mol_type = other DNA
atgtggtggagactgtggtggctgctgctgctgctgctgctgctgtggcccatggtgtgggccgcc

SEQ ID NO: 55 - protein, 23 aa, synthetic construct
  REGION 1..23: note = Description of Artificial Sequence: Synthetic peptide
MWWRLWWLLLLLLLLWPMVWAAA

SEQ ID NO: 56 - DNA, 69 bp, synthetic construct
  misc_feature 1..69: note = Description of Artificial Sequence: Synthetic oligonucleotide
  source 1..69: mol_type = other DNA
atgtggtggagactgtggtggctgctgctgctgctgctgctgctgtggcccatggtgtgggccgccgcc

SEQ ID NO: 57 - DNA, 24 bp, synthetic construct
  misc_feature 1..24: note = Description of Artificial Sequence: Synthetic oligonucleotide
  source 1..24: mol_type = other DNA
taattagctgagtagataagtgat

SEQ ID NO: 58 - DNA, 30 bp, synthetic construct
  misc_feature 1..30: note = Description of Artificial Sequence: Synthetic oligonucleotide
  source 1..30: mol_type = other DNA
ctaggttgttatctccatttagaacaaaat

SEQ ID NO: 59 - protein, 50 aa, synthetic construct
  REGION 1..50: note = Description of Artificial Sequence: Synthetic polypeptide
  VARIANT 1..50: note = MISC_FEATURE - This sequence may encompass 1-10 GGGGS repeating units
GGGGSGGGGSGGGGSGGGGSGGGGSGGGGSGGGGSGGGGSGGGGSGGGGS

SEQ ID NO: 60 - protein, 6 aa, synthetic construct
  REGION 1..6: note = Description of Artificial Sequence: Synthetic peptide
GSGGAP

SEQ ID NO: 61 - protein, 11 aa, synthetic construct
  REGION 1..11: note = Description of Artificial Sequence: Synthetic peptide
TPLGDTTHTSG

SEQ ID NO: 62 - DNA, 19 bp, synthetic construct
  misc_feature 1..19: note = Description of Artificial Sequence: Synthetic oligonucleotide
  source 1..19: mol_type = other DNA
cccatctttacaggctccc

SEQ ID NO: 63 - DNA, 19 bp, synthetic construct
  misc_feature 1..19: note = Description of Artificial Sequence: Synthetic oligonucleotide
  source 1..19: mol_type = other DNA
tctctccctgcaggatact

SEQ ID NO: 64 - DNA, 19 bp, synthetic construct
  misc_feature 1..19: note = Description of Artificial Sequence: Synthetic oligonucleotide
  source 1..19: mol_type = other DNA
ctttttcatacaggaggaa

SEQ ID NO: 65 - DNA, 19 bp, synthetic construct
  misc_feature 1..19: note = Description of Artificial Sequence: Synthetic oligonucleotide
  source 1..19: mol_type = other DNA
tctttatttccaggcaaag

SEQ ID NO: 66 - skipped

SEQ ID NO: 67 - DNA, 21 bp, synthetic construct
  misc_feature 1..21: note = Description of Artificial Sequence: Synthetic oligonucleotide
  source 1..21: mol_type = other DNA
tttcattatttttattataag

SEQ ID NO: 68 - DNA, 21 bp, synthetic construct
  misc_feature 1..21: note = Description of Artificial Sequence: Synthetic oligonucleotide
  source 1..21: mol_type = other DNA
tttccttcttttttttttcag

SEQ ID NO: 69 - DNA, 21 bp, synthetic construct
  misc_feature 1..21: note = Description of Artificial Sequence: Synthetic oligonucleotide
  source 1..21: mol_type = other DNA
tttccttcttttttttttaag

SEQ ID NO: 70 - DNA, 21 bp, synthetic construct
  misc_feature 1..21: note = Description of Artificial Sequence: Synthetic oligonucleotide
  source 1..21: mol_type = other DNA
tttccttctttttattataag

SEQ ID NO: 71 - DNA, 21 bp, synthetic construct
  misc_feature 1..21: note = Description of Artificial Sequence: Synthetic oligonucleotide
  source 1..21: mol_type = other DNA
tttcattattttttttttcag